European Patent Specification EP 3 691 647 B1, published May 27, 2026. Title: New treatment of SMA. Applicant: F. Hoffmann-La Roche AG. The sequence listing filed with the application follows.

SEQUENCE LISTING (9 sequences)

SEQ ID NO: 1 - DNA, 17 bp, Homo sapiens
cccccaaggtgctgcta

SEQ ID NO: 2 - DNA, 21 bp, Homo sapiens
tgaactggaagcaaaggagaa

SEQ ID NO: 3 - DNA, 20 bp, Homo sapiens
ctttcttctgcaggaccagg

SEQ ID NO: 4 - DNA, 20 bp, Homo sapiens
gaaggtgaaggtcggagtca

SEQ ID NO: 5 - DNA, 24 bp, Homo sapiens
aaccatgtagttgaggtcaatgaa

SEQ ID NO: 6 - DNA, 8 bp, Homo sapiens
ttgatggc

SEQ ID NO: 7 - DNA, 17 bp, Homo sapiens
cccccaaggtgctgcta

SEQ ID NO: 8 - DNA, 21 bp, Homo sapiens
tgaactggaagcaaaggacac

SEQ ID NO: 9 - DNA, 20 bp, Homo sapiens
cttccttctgcagggccagg